European Patent Application EP 4 488 294 A1, published January 8, 2025. Title: HER3 BINDING PROTEIN AND USE THEREOF. Applicant: SICHUAN KELUN-BIOTECH BIOPHARMACEUTICAL CO., LTD. Application CN PCT/CN2023/078774, filed February 28, 2023. The sequence listing filed with the application follows.

SEQUENCE LISTING (72 sequences)

SEQ ID NO: 1 - protein, 123 aa, synthetic construct
  source 1..123: note; note (original language) = 22B6D2 VH amino acid sequence
EVHLVESGGGVVQPGRSLRLSCATSGFTFRSYGMHWVRQAPGKGLEWVAVIWYDGSNKYYADSVKGRFTISRDISKNTLYLQMNSLTAEDTAVYYCARYYYDSNGYYDAFDIWGQGTMVTVSS

SEQ ID NO: 2 - protein, 107 aa, synthetic construct
  source 1..107: note; note (original language) = 22B6D2 VL amino acid sequence
DIQLTQSPSFLSASVGDRVTITCRASQGISNYLAWYQQKPGKAPKLLIFAASTLQSGVPSRFSGSGSGAEFTLTISSLEPEDFATYYCQQLNSYPITFGQGTRLEIK

SEQ ID NO: 3 - protein, 128 aa, synthetic construct
  source 1..128: note; note (original language) = 44A4A11 VH amino acid sequence
EVQLLESGGGLVQPGGSLRLSCAASGFTFSSYAMNWVRQAPGKGLEWVSSISDSGGSTYYADSVKGRFTISRDNSKNTLYLQMNSLRAEDTAVYYCAKDGGISMVRGVIIEEGYFDLWGRGTLVTSPQ

SEQ ID NO: 4 - protein, 107 aa, synthetic construct
  source 1..107: note; note (original language) = 44A4A11 VL amino acid sequence
DIQLTQSPSFLSASVGDRVTITCRASQGISSYLAWYQQKPGKAPKLLIYVVSTLQSGVPSRFSGSGSGTEFTLTISSLQPEDFATYYCHQLNSYPLTFGGGTKVEIK

SEQ ID NO: 5 - protein, 124 aa, synthetic construct
  source 1..124: note; note (original language) = 47A3E3 VH amino acid sequence
EVQLQESGPGLVKPSQTLSLTCAISGDSVSSSQSTWNWIRQSPSRGLEWLGRTFYRSRWYNDYALSMKSRITINPDTSKNQFSLQLNPVTPEDTAVYYCARDTYYYGSGGFDYWGQGSRVTVSS

SEQ ID NO: 6 - protein, 106 aa, synthetic construct
  source 1..106: note; note (original language) = 47A3E3 VL amino acid sequence
DIQMTQSPSTLSASVGDRVTITCRASQSLSRWLAWYQQKPEKAPKLLIYKASSLESGVPSRFSGSGSGTEFTLTISTLQPDDFATYYCQQYKNYYSFGQGTKLEIK

SEQ ID NO: 7 - protein, 116 aa, synthetic construct
  source 1..116: note; note (original language) = 100H7D3 VH amino acid sequence
EVQLVESGGGVVLPGRSLRLSCAASGFTFSRNAMHWVRQAPGKGLEWVAVIWHDGSNKYYGDSVKGRFTISRDNSKNTLYLQMDSLTAEDTAVYYCARDRGASDFRGQGTLVTVSS

SEQ ID NO: 8 - protein, 107 aa, synthetic construct
  source 1..107: note; note (original language) = 100H7D3 VL amino acid sequence
DIQMTQSPSTLSASVGDRVTITCRASQSINNWLAWYQQKPEKAPKLLIYKASSLESGVPSRFSGSGSGTEFTLTISSLQPDDFATYYCQQYNSYSLTFGGGTKVEIK

SEQ ID NO: 9 - protein, 8 aa, synthetic construct
  source 1..8: note = 22B6D2 VH CDR1(IMGT)
GFTFRSYG

SEQ ID NO: 10 - protein, 8 aa, synthetic construct
  source 1..8: note = 22B6D2 VH CDR2(IMGT )
IWYDGSNK

SEQ ID NO: 11 - protein, 16 aa, synthetic construct
  source 1..16: note = 22B6D2 VH CDR3(IMGT )
ARYYYDSNGYYDAFDI

SEQ ID NO: 12 - protein, 5 aa, synthetic construct
  source 1..5: note = 22B6D2 VH CDR1(Kabat )
SYGMH

SEQ ID NO: 13 - protein, 17 aa, synthetic construct
  source 1..17: note = 22B6D2 VH CDR2(Kabat )
VIWYDGSNKYYADSVKG

SEQ ID NO: 14 - protein, 14 aa, synthetic construct
  source 1..14: note = 22B6D2 VH CDR3(Kabat )
YYYDSNGYYDAFDI

SEQ ID NO: 15 - protein, 7 aa, synthetic construct
  source 1..7: note = 22B6D2 VH CDR1(Chothia )
GFTFRSY

SEQ ID NO: 16 - protein, 6 aa, synthetic construct
  source 1..6: note = 22B6D2 VH CDR2(Chothia )
WYDGSN

SEQ ID NO: 17 - protein, 14 aa, synthetic construct
  source 1..14: note = 22B6D2 VH CDR3(Chothia )
YYYDSNGYYDAFDI

SEQ ID NO: 18 - protein, 6 aa, synthetic construct
  source 1..6: note = 22B6D2 VL CDR1(IMGT )
QGISNY

SEQ ID NO: 19 - skipped

SEQ ID NO: 20 - protein, 9 aa, synthetic construct
  source 1..9: note = 22B6D2 VL CDR3(IMGT )
QQLNSYPIT

SEQ ID NO: 21 - protein, 11 aa, synthetic construct
  source 1..11: note = 22B6D2 VL CDR1(Kabat /Chothia )
RASQGISNYLA

SEQ ID NO: 22 - protein, 7 aa, synthetic construct
  source 1..7: note = 22B6D2 VL CDR2(Kabat Chothia )
AASTLQS

SEQ ID NO: 23 - protein, 9 aa, synthetic construct
  source 1..9: note = 22B6D2 VL CDR3(Kabat/Chothia )
QQLNSYPIT

SEQ ID NO: 24 - protein, 8 aa, synthetic construct
  source 1..8: note = 44A4A11 VH CDR1(IMGT )
GFTFSSYA

SEQ ID NO: 25 - protein, 8 aa, synthetic construct
  source 1..8: note = 44A4A11 VH CDR2(IMGT )
ISDSGGST

SEQ ID NO: 26 - protein, 21 aa, synthetic construct
  source 1..21: note = 44A4A11 VH CDR3(IMGT )
AKDGGISMVRGVIIEEGYFDL

SEQ ID NO: 27 - protein, 5 aa, synthetic construct
  source 1..5: note = 44A4A11 VH CDR1(Kabat )
SYAMN

SEQ ID NO: 28 - protein, 17 aa, synthetic construct
  source 1..17: note = 44A4A11 VH CDR2(Kabat )
SISDSGGSTYYADSVKG

SEQ ID NO: 29 - protein, 19 aa, synthetic construct
  source 1..19: note = 44A4A11 VH CDR3(Kabat/Chothia )
DGGISMVRGVIIEEGYFDL

SEQ ID NO: 30 - protein, 7 aa, synthetic construct
  source 1..7: note = 44A4A11 VH CDR1(Chothia )
GFTFSSY

SEQ ID NO: 31 - protein, 6 aa, synthetic construct
  source 1..6: note = 44A4A11 VH CDR2(Chothia )
SDSGGS

SEQ ID NO: 32 - protein, 6 aa, synthetic construct
  source 1..6: note = 47A3E3 VL CDR1(IMGT )
QSLSRW

SEQ ID NO: 33 - skipped

SEQ ID NO: 34 - protein, 8 aa, synthetic construct
  source 1..8: note = 47A3E3 VL CDR3(IMGT/Kabat/Chothia )
QQYKNYYS

SEQ ID NO: 35 - protein, 11 aa, synthetic construct
  source 1..11: note = 47A3E3 VL CDR1(Kabat/Chothia )
RASQSLSRWLA

SEQ ID NO: 36 - protein, 7 aa, synthetic construct
  source 1..7: note = 47A3E3/100H7D3 VL CDR2(Kabat/Chothia )
KASSLES

SEQ ID NO: 37 - protein, 10 aa, synthetic construct
  source 1..10: note = 47A3E3 VH CDR1(IMGT )
GDSVSSSQST

SEQ ID NO: 38 - protein, 9 aa, synthetic construct
  source 1..9: note = 47A3E3 VH CDR2(IMGT )
TFYRSRWYN

SEQ ID NO: 39 - protein, 14 aa, synthetic construct
  source 1..14: note = 47A3E3 VH CDR3(IMGT )
ARDTYYYGSGGFDY

SEQ ID NO: 40 - protein, 7 aa, synthetic construct
  source 1..7: note = 47A3E3 VH CDR1(Kabat )
SSQSTWN

SEQ ID NO: 41 - protein, 18 aa, synthetic construct
  source 1..18: note = 47A3E3 VH CDR2(Kabat )
RTFYRSRWYNDYALSMKS

SEQ ID NO: 42 - protein, 12 aa, synthetic construct
  source 1..12: note = 47A3E3 VH CDR3(Kabat/Chothia )
DTYYYGSGGFDY

SEQ ID NO: 43 - protein, 9 aa, synthetic construct
  source 1..9: note = 47A3E3 VH CDR1(Chothia )
GDSVSSSQS

SEQ ID NO: 44 - protein, 7 aa, synthetic construct
  source 1..7: note = 47A3E3 VH CDR2(Chothia )
FYRSRWY

SEQ ID NO: 45 - protein, 8 aa, synthetic construct
  source 1..8: note = 100H7D3 VH CDR1(IMGT )
GFTFSRNA

SEQ ID NO: 46 - protein, 8 aa, synthetic construct
  source 1..8: note = 100H7D3 VH CDR2(IMGT )
IWHDGSNK

SEQ ID NO: 47 - protein, 9 aa, synthetic construct
  source 1..9: note = 100H7D3 VH CDR3(IMGT )
ARDRGASDF

SEQ ID NO: 48 - protein, 5 aa, synthetic construct
  source 1..5: note = 100H7D3 VH CDR1(Kabat )
RNAMH

SEQ ID NO: 49 - protein, 17 aa, synthetic construct
  source 1..17: note = 100H7D3 VH CDR2(Kabat )
VIWHDGSNKYYGDSVKG

SEQ ID NO: 50 - protein, 7 aa, synthetic construct
  source 1..7: note = 100H7D3 VH CDR3(Kabat/Chothia )
DRGASDF

SEQ ID NO: 51 - protein, 7 aa, synthetic construct
  source 1..7: note = 100H7D3 VH CDR1(Chothia )
GFTFSRN

SEQ ID NO: 52 - protein, 6 aa, synthetic construct
  source 1..6: note = 100H7D3 VH CDR2(Chothia )
WHDGSN

SEQ ID NO: 53 - protein, 6 aa, synthetic construct
  source 1..6: note = 100H7D3 VL CDR1(IMGT )
QSINNW

SEQ ID NO: 54 - protein, 9 aa, synthetic construct
  source 1..9: note = 100H7D3 VL CDR3(IMGT/Kabat/Chothia )
QQYNSYSLT

SEQ ID NO: 55 - DNA, 369 bp, synthetic construct
  source 1..369: mol_type = other DNA; note; note (original language) = 22B6D2 VH nucleotide sequence
gaagtgcatctagtggaaagtggtggtggtgtggtgcagcctggacggagcctgcggctgtcttgtgccacatctggcttcaccttcagatcctacggcatgcactgggtgcggcaggctcccggtaagggcctggaatgggtggccgtcatctggtatgacggctctaacaagtactacgccgattccgtgaaaggcagattcacaatctctagagacatctccaagaacaccctgtacctgcagatgaactccctgaccgctgaggacaccgccgtgtactactgcgccagatactactacgactccaatggctactacgatgcttttgacatctggggccaaggcaccatggtgaccgtgtccagc

SEQ ID NO: 56 - DNA, 321 bp, synthetic construct
  source 1..321: mol_type = other DNA; note; note (original language) = 22B6D2 VL nucleotide sequence
gatattcaactaactcaaagtccaagttttctgtccgcctccgtgggcgatagagtgaccatcacctgtagagccagccaaggcatctccaactacctggcctggtaccagcagaagcctggcaaagctccaaagctgctcatctttgctgcttctacactgcagtccggcgtgccttctcggttctccggatctggatctggcgccgagttcacactgaccatcagctctctggaacctgaggacttcgccacctactactgccagcagctgaactcctatcccatcaccttcggccagggcacccggctggagatcaag

SEQ ID NO: 57 - DNA, 384 bp, synthetic construct
  source 1..384: mol_type = other DNA; note; note (original language) = 44A4A11 VH nucleotide sequence
gaagtgcaactgttggaaagtgggggtggtttggttcagcctggtggttcattgagattgtcttgcgccgctagtggatttacattctcctcctacgcaatgaactgggttcgccaggcccctggtaaaggactggagtgggtgtcttctatctctgactcaggcggttcaacatattatgcagattctgtgaaggggagatttacaattagccgggacaactctaaaaatactctgtacctgcagatgaactccctgagagcagaggatacagcagtttactactgcgctaaagacggaggaatcagtatggtgagaggcgtcattattgaggagggatattttgatttgtggggcagagggacactcgtgacctccccacag

SEQ ID NO: 58 - DNA, 321 bp, synthetic construct
  source 1..321: mol_type = other DNA; note; note (original language) = 44A4A11 VL nucleotide sequence
gatatacagttgactcagagcccttcctttttgtccgcttctgtcggagatagagtgactatcacctgtagggcctctcaaggaatttccagttatcttgcctggtatcagcagaaacccggcaaggctcccaaactcctgatctacgtggtgagcacgctgcagtctggagtccctagcaggttcagcggcagcgggtctgggaccgaatttactctgacaatctcttccctccagcctgaagattttgctacatactactgccatcaattgaattcctatccattgacctttggcggcggtaccaaggtggagatcaag

SEQ ID NO: 59 - DNA, 372 bp, synthetic construct
  source 1..372: mol_type = other DNA; note; note (original language) = 47A3E3 VH nucleotide sequence
gaggtgcagctgcaggagtctggaccaggcctggtgaagccatctcagaccctgtccctgacatgcgccatcagcggcgactctgtgtccagctctcagtctacctggaactggatcagacagtctccatctagaggcctggagtggctgggaaggacattctataggtcccggtggtataatgactacgctctgtccatgaagagccggatcaccatcaacccagatacaagcaagaatcagttttctctgcagctgaaccccgtgacccctgaggacacagccgtgtactattgtgctagagatacctactattacggctccggcggcttcgattactggggccagggcagccgcgtgacagtgtccagc

SEQ ID NO: 60 - DNA, 318 bp, synthetic construct
  source 1..318: mol_type = other DNA; note; note (original language) = 47A3E3 VL nucleotide sequence
gatattcaaatgactcaaagtccaagtactctgtctgcttccgtgggcgacagagtgaccatcacctgtcgggcctctcagtccctgtccagatggctggcctggtaccagcaaaaacctgagaaggctcctaagctgctgatctacaaggcctcctctctggaatccggcgtgcccagccggtttagcggatctggctctggcaccgagttcaccctgaccatctccacactgcagcctgatgacttcgccacctactactgccagcagtacaagaactactattccttcggccagggcaccaagctcgagatcaag

SEQ ID NO: 61 - DNA, 348 bp, synthetic construct
  source 1..348: mol_type = other DNA; note; note (original language) = 100H7D3 VH nucleotide sequence
gaggtgcagctggtggagtccggcggcggcgtggtgctgcctggaagatctctgagactgtcctgtgctgcttctggattcaccttttccagaaatgctatgcactgggtcagacaggctccaggaaagggcctggagtgggtggctgtgatctggcatgacggcagcaataagtactatggcgattctgtgaagggcaggttcaccatctctcgggacaactccaagaatacactgtacctgcagatggactccctgaccgccgaggatacagctgtgtactattgtgccagggaccggggcgctagcgattttaggggccagggcaccctggtgacagtgtccagc

SEQ ID NO: 62 - DNA, 321 bp, synthetic construct
  source 1..321: mol_type = other DNA; note; note (original language) = 100H7D3 VL nucleotide sequence
gacatccagatgacccagtctccttctacactgtctgcttctgtgggcgatagggtgaccatcacatgccgggcctctcagtccatcaacaattggctggcttggtaccagcagaagcccgagaaggcccctaagctgctgatctataaggcttccagcctggagtccggcgtgccatctagattctctggctctggctccggaaccgagtttaccctgacaatctcttccctgcagcccgacgatttcgctacatactattgtcagcagtacaacagctattctctgacctttgggggagggacaaaggtggagatcaag

SEQ ID NO: 63 - protein, 330 aa, synthetic construct
  source 1..330: note; note (original language) = IgG1 heavy chain constant region amino acid sequence
ASTKGPSVFPLAPSSKSTSGGTAALGCLVKDYFPEPVTVSWNSGALTSGVHTFPAVLQSSGLYSLSSVVTVPSSSLGTQTYICNVNHKPSNTKVDKRVEPKSCDKTHTCPPCPAPELLGGPSVFLFPPKPKDTLMISRTPEVTCVVVDVSHEDPEVKFNWYVDGVEVHNAKTKPREEQYNSTYRVVSVLTVLHQDWLNGKEYKCKVSNKALPAPIEKTISKAKGQPREPQVYTLPPSREEMTKNQVSLTCLVKGFYPSDIAVEWESNGQPENNYKTTPPVLDSDGSFFLYSKLTVDKSRWQQGNVFSCSVMHEALHNHYTQKSLSLSPGK

SEQ ID NO: 64 - DNA, 993 bp, synthetic construct
  source 1..993: mol_type = other DNA; note; note (original language) = IgG1 heavy chain constant region nucleotide sequence
gcctctacaaagggcccatctgtctttcccctggccccttcttccaagtctacctccggcggcaccgctgctctgggctgcctggtgaaggactacttccctgagcctgtgaccgtgtcttggaacagcggtgctctgacctctggcgtgcacaccttccccgccgtactgcagtcctctggcctgtacagcctttcctccgtggtgaccgttccttcttcctctctgggcacacagacctacatctgcaacgtgaatcacaagccttctaacaccaaggtggacaagcgggtggaacccaagtcctgcgataaaacccacacatgtcctccatgccctgcccctgagctgctgggcggccctagcgtgttcctgttccctcctaaacctaaggacaccctgatgatcagccggacacctgaagtgacctgtgtggtggtggatgtgtctcatgaggaccccgaagtgaaattcaactggtatgtggatggcgtggaagtgcacaacgctaaaaccaagcccagagaggaacagtacaattccacatatagagtggtctctgtgctgaccgtgctgcaccaggactggctgaacgggaaagagtacaagtgcaaggtcagcaacaaggctctgcctgctcctatcgaaaagaccatctccaaggccaagggacagccacgggagcctcaggtgtacaccctgcctccatccagagaagagatgaccaagaaccaggtgtccctgacctgcctggtgaagggcttctacccttccgacatcgccgtcgagtgggagagcaacggccagccagagaacaactacaagaccacgcctcctgttctggactccgacggctccttttttctgtactccaagctgacagtggacaagagccgctggcagcagggcaacgtgttctcctgttctgtgatgcacgaggctctccataaccactacacccagaagtctctgtccctgtcccctggcaagtga

SEQ ID NO: 65 - protein, 107 aa, synthetic construct [sequence omitted]

SEQ ID NO: 66 - DNA, 324 bp, synthetic construct
  source 1..324: mol_type = other DNA; note; note (original language) = Light chain constant region nucleotide sequence
cggaccgtggccgctccttctgtgttcatctttcctccttccgacgagcagctgaagtctggcaccgccagcgtcgtttgtctgctgaacaacttctaccctagagaggccaaggtgcagtggaaagtggacaatgctctgcaatccggcaactcccaagagtccgtgaccgaacaggactccaaggactctacctattccctctcctccaccctgacactgtccaaagccgactacgagaagcacaaggtgtacgcctgcgaagtgacccaccagggcctgtcttctccagtgacaaagtccttcaaccggggcgagtgctga

SEQ ID NO: 67 - protein, 6 aa, synthetic construct
  source 1..6: note = 44A4A11 VL CDR1(IMGT )
QGISSY

SEQ ID NO: 68 - skipped

SEQ ID NO: 69 - protein, 9 aa, synthetic construct
  source 1..9: note; note (original language) = 44A4A11 VL CDR3(IMGT/Kabat/Chothia )
HQLNSYPLT

SEQ ID NO: 70 - protein, 11 aa, synthetic construct
  source 1..11: note = 44A4A11 VL CDR1(Kabat/Chothia )
RASQGISSYLA

SEQ ID NO: 71 - protein, 7 aa, synthetic construct
  source 1..7: note = 44A4A11 VL CDR2(Kabat/Chothia )
VVSTLQS

SEQ ID NO: 72 - protein, 11 aa, synthetic construct
  source 1..11: note = 100H7D3 VL CDR1(Kabat/Chothia )
RASQSINNWLA